European Patent Application EP 4 116 421 A1, published January 11, 2023. Title: Construct of self-circularization RNA. Applicant: Rznomics Inc. The sequence listing filed with the application follows.

SEQUENCE LISTING (43 sequences)

SEQ ID NO: 1 - RNA, 6 nt, Artificial Sequence
  IGS region of self-circulariztion RNA
  variation (2)..(6): N is any one of A, G, U, and C
gnnnnn

SEQ ID NO: 2 - RNA, 6 nt, Artificial Sequence
  target site region of self-circulariztion RNA
  variation (1)..(5): N is any one of A, G, U, and C
nnnnnu

SEQ ID NO: 3 - DNA, 20 bp, Artificial Sequence
  T7 promoter
taatacgactcactataggg

SEQ ID NO: 4 - DNA, 150 bp, Artificial Sequence
  AS 150: AS region of expression vector for self-circulariztion RNA
ggcggccagcatggagaactgccatggctcagccaggtagtactgtgggtactcgaagtggctgcgtaccacacccgtcgcattggagaagggcacgtagaagttagggccttctgtgccattcatggctgtggcccttgtggctgaccc

SEQ ID NO: 5 - DNA, 6 bp, Artificial Sequence
  IGS region of expression vector for self-circulariztion RNA
gcccaa

SEQ ID NO: 6 - DNA, 387 bp, Artificial Sequence
  ribozyme region of expression vector for self-circulariztion RNA
aaaagttatcaggcatgcacctggtagctagtctttaaaccaatagattgcatcggtttaaaaggcaagaccgtcaaattgcgggaaaggggtcaacagccgttcagtaccaagtctcaggggaaactttgagatggccttgcaaagggtatggtaataagctgacggacatggtcctaaccacgcagccaagtcctaagtcaacagatcttctgttgatatggatgcagttcacagactaaatgtcggtcggggaagatgtattcttctcataagatatagtcggacctctccttaatgggagctagcggatgaagtgatgcaacactggagccgctgggaactaatttgtatgcgaaagtatattgattagttttggagtactcg

SEQ ID NO: 7 - DNA, 463 bp, Artificial Sequence
  EMCV IRES region of expression vector for self-circulariztion RNA
gagggcccggaaacctggccctgtcttcttgacgagcattcctaggggtctttcccctctcgccaaaggaatgcaaggtctgttgaatgtcgtgaaggaagcagttcctctggaagcttcttgaagacaaacaacgtctgtagcgaccctttgcaggcagcggaaccccccacctggcgacaggtgcctctgcggccaaaagccacgtgtataagatacacctgcaaaggcggcacaaccccagtgccacgttgtgagttggatagttgtggaaagagtcaaatggctctcctcaagcgtattcaacaaggggctgaaggatgcccagaaggtaccccattgtatgggatctgatctggggcctcggtgcacatgctttacatgtgtttagtcgaggttaaaaaaacgtctaggccccccgaaccacggggacgtggttttcctttgaaaaacacgatgataa

SEQ ID NO: 8 - DNA, 558 bp, Artificial Sequence
  transgene region of expression vector for self-circulariztion RNA: Gaussia Luciferase
atgggagtcaaagttctgtttgccctgatctgcatcgctgtggccgaggccaagcccaccgagaacaacgaagacttcaacatcgtggccgtggccagcaacttcgcgaccacggatctcgatgctgaccgcgggaagttgcccggcaagaagctgccgctggaggtgctcaaagagatggaagccaatgcccggaaagctggctgcaccaggggctgtctgatctgcctgtcccacatcaagtgcacgcccaagatgaagaagttcatcccaggacgctgccacacctacgaaggcgacaaagagtccgcacagggcggcataggcgaggcgatcgtcgacattcctgagattcctgggttcaaggacttggagcccatggagcagttcatcgcacaggtcgatctgtgtgtggactgcacaactggctgcctcaaagggcttgccaacgtgcagtgttctgacctgctcaagaagtggctgccgcaacgctgtgcgacctttgccagcaagatccagggccaggtggacaagatcaagggggccggtggtgactaa

SEQ ID NO: 9 - DNA, 150 bp, Artificial Sequence
  ABS region of expression vector for self-circulariztion RNA
gggtcagccacaagggccacagccatgaatggcacagaaggccctaacttctacgtgcccttctccaatgcgacgggtgtggtacgcagccacttcgagtacccacagtactacctggctgagccatggcagttctccatgctggccgcc

SEQ ID NO: 10 - DNA, 1908 bp, Artificial Sequence
  DNA template encoding self-circularizaion RNA of the example 1
gggattcgaacatcgattaatacgactcactataggggcatcgattgaattgtcgacgaattcggcggccagcatggagaactgccatggctcagccaggtagtactgtgggtactcgaagtggctgcgtaccacacccgtcgcattggagaagggcacgtagaagttagggccttctgtgccattcatggctgtggcccttgtggctgacccgaattccgtactccgcccaaaaaagttatcaggcatgcacctggtagctagtctttaaaccaatagattgcatcggtttaaaaggcaagaccgtcaaattgcgggaaaggggtcaacagccgttcagtaccaagtctcaggggaaactttgagatggccttgcaaagggtatggtaataagctgacggacatggtcctaaccacgcagccaagtcctaagtcaacagatcttctgttgatatggatgcagttcacagactaaatgtcggtcggggaagatgtattcttctcataagatatagtcggacctctccttaatgggagctagcggatgaagtgatgcaacactggagccgctgggaactaatttgtatgcgaaagtatattgattagttttggagtactcgcgagtacgcttaagaaaaaaaaaagagggcccggaaacctggccctgtcttcttgacgagcattcctaggggtctttcccctctcgccaaaggaatgcaaggtctgttgaatgtcgtgaaggaagcagttcctctggaagcttcttgaagacaaacaacgtctgtagcgaccctttgcaggcagcggaaccccccacctggcgacaggtgcctctgcggccaaaagccacgtgtataagatacacctgcaaaggcggcacaaccccagtgccacgttgtgagttggatagttgtggaaagagtcaaatggctctcctcaagcgtattcaacaaggggctgaaggatgcccagaaggtaccccattgtatgggatctgatctggggcctcggtgcacatgctttacatgtgtttagtcgaggttaaaaaaacgtctaggccccccgaaccacggggacgtggttttcctttgaaaaacacgatgataagcttgccacaacccttaagaccggtatgggagtcaaagttctgtttgccctgatctgcatcgctgtggccgaggccaagcccaccgagaacaacgaagacttcaacatcgtggccgtggccagcaacttcgcgaccacggatctcgatgctgaccgcgggaagttgcccggcaagaagctgccgctggaggtgctcaaagagatggaagccaatgcccggaaagctggctgcaccaggggctgtctgatctgcctgtcccacatcaagtgcacgcccaagatgaagaagttcatcccaggacgctgccacacctacgaaggcgacaaagagtccgcacagggcggcataggcgaggcgatcgtcgacattcctgagattcctgggttcaaggacttggagcccatggagcagttcatcgcacaggtcgatctgtgtgtggactgcacaactggctgcctcaaagggcttgccaacgtgcagtgttctgacctgctcaagaagtggctgccgcaacgctgtgcgacctttgccagcaagatccagggccaggtggacaagatcaagggggccggtggtgactaaaaaaaaaaaaaccggtttgggtgggagcagccacgggtcagccacaagggccacagccatgaatggcacagaaggccctaacttctacgtgcccttctccaatgcgacgggtgtggtacgcagccacttcgagtacccacagtactacctggctgagccatggcagttctccatgctggccgccaagcttgcctcgagcagcgctgctcgagagatct

SEQ ID NO: 11 - DNA, 56 bp, Artificial Sequence
  T7 Circular Forward primer
gggattcgaacatcgattaatacgactcactataggggcatcgattgaattgtcga

SEQ ID NO: 12 - DNA, 34 bp, Artificial Sequence
  T7 Circular Reverse primer
agatctctcgagcagcgctgctcgaggcaagctt

SEQ ID NO: 13 - DNA, 21 bp, Artificial Sequence
  Circular STS Forward primer of the example 2-2
ccctgagtggctgagctcagg

SEQ ID NO: 14 - DNA, 23 bp, Artificial Sequence
  Circular STS Reverse primer of the example 2-2
cagcaagcatactaaattgccag

SEQ ID NO: 15 - DNA, 25 bp, Artificial Sequence
  Circular STS Forward primer of the example 3
caaggacttggagcccatggagcag

SEQ ID NO: 16 - DNA, 23 bp, Artificial Sequence
  Circular STS Reverse primer 2 of the example 3
tgtgccgcctttgcaggtgtatc

SEQ ID NO: 17 - DNA, 50 bp, Artificial Sequence
  DNA sequecne for AS50 region
aagttagggccttctgtgccattcatggctgtggcccttgtggctgaccc

SEQ ID NO: 18 - DNA, 100 bp, Artificial Sequence
  DNA sequecne for AS100 region
actcgaagtggctgcgtaccacacccgtcgcattggagaagggcacgtagaagttagggccttctgtgccattcatggctgtggcccttgtggctgaccc

SEQ ID NO: 19 - DNA, 150 bp, Artificial Sequence; identical to SEQ ID NO: 4
  DNA sequecne for AS150 region

SEQ ID NO: 20 - DNA, 200 bp, Artificial Sequence
  DNA sequecne for AS200 region
agcgtgaggaagttgatggggaagcccagcacgatcagcagaaacatgtaggcggccagcatggagaactgccatggctcagccaggtagtactgtgggtactcgaagtggctgcgtaccacacccgtcgcattggagaagggcacgtagaagttagggccttctgtgccattcatggctgtggcccttgtggctgaccc

SEQ ID NO: 21 - DNA, 250 bp, Artificial Sequence
  DNA sequecne for AS250 region
ggatgtagttgagaggcgtgcgcagcttcttgtgctggacggtgacgtagagcgtgaggaagttgatggggaagcccagcacgatcagcagaaacatgtaggcggccagcatggagaactgccatggctcagccaggtagtactgtgggtactcgaagtggctgcgtaccacacccgtcgcattggagaagggcacgtagaagttagggccttctgtgccattcatggctgtggcccttgtggctgaccc

SEQ ID NO: 22 - DNA, 300 bp, Artificial Sequence
  DNA sequecne for AS300 region
ggtgaagccacctaggaccatgaagaggtcagccacggctaggttgagcaggatgtagttgagaggcgtgcgcagcttcttgtgctggacggtgacgtagagcgtgaggaagttgatggggaagcccagcacgatcagcagaaacatgtaggcggccagcatggagaactgccatggctcagccaggtagtactgtgggtactcgaagtggctgcgtaccacacccgtcgcattggagaagggcacgtagaagttagggccttctgtgccattcatggctgtggcccttgtggctgaccc

SEQ ID NO: 23 - DNA, 10 bp, Artificial Sequence
  DNA sequecne for A10: spacer region
aaaaaaaaaa

SEQ ID NO: 24 - DNA, 30 bp, Artificial Sequence
  DNA sequecne for A30: spacer region
aaaaaaaaaaaaaaaaaaaaaaaaaaaaaa

SEQ ID NO: 25 - DNA, 39 bp, Artificial Sequence
  DNA sequecne for A50: spacer region
aaaaaaaaaaaaaaaaaaaaaaaaaaaaaaaaaaaaaaa

SEQ ID NO: 26 - DNA, 35 bp, Artificial Sequence
  DNA sequecne for control 1: spacer region
ggtagtggtgctactaacttcagcctgctgaagca

SEQ ID NO: 27 - DNA, 34 bp, Artificial Sequence
  DNA sequecne for control 2: spacer region
ggtagtaaactactaactacaacctgctgaagca

SEQ ID NO: 28 - DNA, 6 bp, Artificial Sequence
  Aat2 site
gacgtc

SEQ ID NO: 29 - DNA, 1522 bp, Artificial Sequence
  DNA template encoding self-circularizaion RNA of the example 7
gggattcgaacatcgattaatacgactcactataggggcccaaaaaagttatcaggcatgcacctggtagctagtctttaaaccaatagattgcatcggtttaaaaggcaagaccgtcaaattgcgggaaaggggtcaacagccgttcagtaccaagtctcaggggaaactttgagatggccttgcaaagggtatggtaataagctgacggacatggtcctaaccacgcagccaagtcctaagtcaacagatcttctgttgatatggatgcagttcacagactaaatgtcggtcggggaagatgtattcttctcataagatatagtcggacctctccttaatgggagctagcggatgaagtgatgcaacactggagccgctgggaactaatttgtatgcgaaagtatattgattagttttggagtactcgcgagtacgcttaagaaaaaaaaaagagggcccggaaacctggccctgtcttcttgacgagcattcctaggggtctttcccctctcgccaaaggaatgcaaggtctgttgaatgtcgtgaaggaagcagttcctctggaagcttcttgaagacaaacaacgtctgtagcgaccctttgcaggcagcggaaccccccacctggcgacaggtgcctctgcggccaaaagccacgtgtataagatacacctgcaaaggcggcacaaccccagtgccacgttgtgagttggatagttgtggaaagagtcaaatggctctcctcaagcgtattcaacaaggggctgaaggatgcccagaaggtaccccattgtatgggatctgatctggggcctcggtgcacatgctttacatgtgtttagtcgaggttaaaaaaacgtctaggccccccgaaccacggggacgtggttttcctttgaaaaacacgatgataagcttgccacaacccttaagaccggtatgggagtcaaagttctgtttgccctgatctgcatcgctgtggccgaggccaagcccaccgagaacaacgaagacttcaacatcgtggccgtggccagcaacttcgcgaccacggatctcgatgctgaccgcgggaagttgcccggcaagaagctgccgctggaggtgctcaaagagatggaagccaatgcccggaaagctggctgcaccaggggctgtctgatctgcctgtcccacatcaagtgcacgcccaagatgaagaagttcatcccaggacgctgccacacctacgaaggcgacaaagagtccgcacagggcggcataggcgaggcgatcgtcgacattcctgagattcctgggttcaaggacttggagcccatggagcagttcatcgcacaggtcgatctgtgtgtggactgcacaactggctgcctcaaagggcttgccaacgtgcagtgttctgacctgctcaagaagtggctgccgcaacgctgtgcgacctttgccagcaagatccagggccaggtggacaagatcaagggggccggtggtgactaaaaaaaaaaaaaccggtttgggt

SEQ ID NO: 30 - RNA, 6 nt, Artificial Sequence
  RZ004 variant of P1 region: internal guide sequence composing P1 helix
gcccaa

SEQ ID NO: 31 - RNA, 6 nt, Artificial Sequence
  RZ004 variant of P1 region: target site composing P1 helix
uugggu

SEQ ID NO: 32 - RNA, 6 nt, Artificial Sequence
  RZ001 variant of P1 region: internal guide sequence composing P1 helix
ggcagg

SEQ ID NO: 33 - RNA, 6 nt, Artificial Sequence
  RZ001 variant of P1 region: target site composing P1 helix
ccugcu

SEQ ID NO: 34 - RNA, 6 nt, Artificial Sequence
  RZ003 variant of P1 region: internal guide sequence composing P1 helix
gcgucc

SEQ ID NO: 35 - RNA, 6 nt, Artificial Sequence
  RZ003 variant of P1 region: target site composing P1 helix
ggacgu

SEQ ID NO: 36 - RNA, 6 nt, Artificial Sequence
  GC rich variant of P1 region: internal guide sequence composing P1 helix
gcgcgc

SEQ ID NO: 37 - RNA, 6 nt, Artificial Sequence
  GC rich variant of P1 region: target site composing P1 helix
gcgcgu

SEQ ID NO: 38 - RNA, 6 nt, Artificial Sequence
  AU rich variant of P1 region: internal guide sequence composing P1 helix
guaaau

SEQ ID NO: 39 - RNA, 6 nt, Artificial Sequence
  AU rich variant of P1 region: target site composing P1 helix
auuuau

SEQ ID NO: 40 - RNA, 6 nt, Artificial Sequence
  2 sites variant of P1 region: internal guide sequence composing P1 helix
guguug

SEQ ID NO: 41 - RNA, 6 nt, Artificial Sequence
  2 sites variant of P1 region: target site composing P1 helix
caacau

SEQ ID NO: 42 - RNA, 6 nt, Artificial Sequence
  No complementary variant of P1 region: internal guide sequence composing P1 helix
gcccaa

SEQ ID NO: 43 - RNA, 6 nt, Artificial Sequence
  No complementary variant of P1 region: target site composing P1 helix
aacccg